European Patent Application EP 4 342 488 A1, published March 27, 2024. Title: Chimeric antigen receptor specific for folate receptor 1. Applicant: Miltenyi Biotec b.V. & Co KG. Application EP EP22197771.3, filed September 26, 2022. The sequence listing filed with the application follows.

SEQUENCE LISTING (113 sequences)

SEQ ID NO: 1 - DNA, 372 bp, synthetic construct
  source 1..372: mol_type = other DNA
gaggtccaactggtggagagcggtggaggtgttgtgcaacctggccggtccctgcgcctgtcctgctccgcatctggcttcaccttcagcggctatgggttgtcttgggtgagacaggcacctggaaaaggtcttgagtgggttgcaatgattagtagtggtggtagttatacctactatgcagacagtgtgaagggtagatttgcaatatcgcgagacaacgccaagaacacattgttcctgcaaatggacagcctgagacccgaagacaccggggtctatttttgtgcaagacatggggacgatcccgcctggttcgcttattggggccaagggaccccggtcaccgtctcctcagcctccaccaagggc

SEQ ID NO: 2 - protein, 124 aa, synthetic construct
EVQLVESGGGVVQPGRSLRLSCSASGFTFSGYGLSWVRQAPGKGLEWVAMISSGGSYTYYADSVKGRFAISRDNAKNTLFLQMDSLRPEDTGVYFCARHGDDPAWFAYWGQGTPVTVSSASTKG

SEQ ID NO: 3 - DNA, 334 bp, synthetic construct
  source 1..334: mol_type = other DNA
gacatccagctgacccagagcccaagcagcctgagcgccagcgtgggtgacagagtgaccatcacctgtagtgtcagctcaagtataagttccaacaacttgcactggtaccagcagaagccaggtaaggctccaaagccatggatctacggcacatccaacctggcttctggtgtgccaagcagattcagcggtagcggtagcggtaccgactacaccttcaccatcagcagcctccagccagaggacatcgccacctactactgccaacagtggagtagttacccgtacatgtacacgttcggccaagggaccaaggtggaaatcaaacgaa

SEQ ID NO: 4 - protein, 112 aa, synthetic construct
DIQLTQSPSSLSASVGDRVTITCSVSSSISSNNLHWYQQKPGKAPKPWIYGTSNLASGVPSRFSGSGSGTDYTFTISSLQPEDIATYYCQQWSSYPYMYTFGQGTKVEIKRT

SEQ ID NO: 5 - DNA, 369 bp, synthetic construct
  source 1..369: mol_type = other DNA
caggtacagctcgtgcagtccggcgccgaggtggtgaagcctggtgccagcgtgaagatctcctgtaaagccagtggatacacattcaccggttattttatgaattgggtgaaacagagcccaggccaatccctcgaatggatagggcgaatccacccatatgacggggacaccttttacaaccagaaattccaggggaaagccactctgacagtggacaagagttccaacactgcacacatggagcttctctccctgaccagcgaagacttcgctgtttattactgtacccgttatgatggttcccgtgcaatggactactggggccaagggaccactgtcaccgtaagttccgccagcaccaagggc

SEQ ID NO: 6 - protein, 123 aa, synthetic construct
QVQLVQSGAEVVKPGASVKISCKASGYTFTGYFMNWVKQSPGQSLEWIGRIHPYDGDTFYNQKFQGKATLTVDKSSNTAHMELLSLTSEDFAVYYCTRYDGSRAMDYWGQGTTVTVSSASTKG

SEQ ID NO: 7 - DNA, 339 bp, synthetic construct
  source 1..339: mol_type = other DNA
gacattgtgctgacacagtcccccctttcactggctgtatccctcggccagcccgctatcatcagctgcaaggcaagccagagcgtgagttttgccggcacttcacttatgcattggtaccatcagaaaccaggccagcaaccaaggctgctgatttatcgggcaagcaacctggaggccggcgtgcccgaccgctttagcgggagcggctccaagactgacttcactctgaccatctcccccgtagaagcagaagatgctgcaacctactactgtcagcagtctcgcgagtatccttatacattcggaggcggaactaaactggagattaaacgtacg

SEQ ID NO: 8 - protein, 113 aa, synthetic construct
DIVLTQSPLSLAVSLGQPAIISCKASQSVSFAGTSLMHWYHQKPGQQPRLLIYRASNLEAGVPDRFSGSGSKTDFTLTISPVEAEDAATYYCQQSREYPYTFGGGTKLEIKRT

SEQ ID NO: 9 - DNA, 15 bp, synthetic construct
  source 1..15: mol_type = other DNA
ggctatgggttgtct

SEQ ID NO: 10 - protein, 5 aa, synthetic construct
GYGLS

SEQ ID NO: 11 - DNA, 51 bp, synthetic construct
  source 1..51: mol_type = other DNA
atgattagtagtggtggtagttatacctactatgcagacagtgtgaagggt

SEQ ID NO: 12 - protein, 17 aa, synthetic construct
MISSGGSYTYYADSVKG

SEQ ID NO: 13 - DNA, 30 bp, synthetic construct
  source 1..30: mol_type = other DNA
catggggacgatcccgcctggtttgcttat

SEQ ID NO: 14 - protein, 11 aa, synthetic construct
HGDDPAWFAYW

SEQ ID NO: 15 - DNA, 36 bp, synthetic construct
  source 1..36: mol_type = other DNA
agtgtcagctcaagtataagttccaacaacttgcac

SEQ ID NO: 16 - protein, 12 aa, synthetic construct
SVSSSISSNNLH

SEQ ID NO: 17 - DNA, 21 bp, synthetic construct
  source 1..21: mol_type = other DNA
ggcacatccaacctggcttct

SEQ ID NO: 18 - protein, 7 aa, synthetic construct
GTSNLAS

SEQ ID NO: 19 - DNA, 27 bp, synthetic construct
  source 1..27: mol_type = other DNA
cagcagtctcgcgagtatccttataca

SEQ ID NO: 20 - protein, 9 aa, synthetic construct
QQSREYPYT

SEQ ID NO: 21 - DNA, 30 bp, synthetic construct
  source 1..30: mol_type = other DNA
ggatacacattcaccggttattttatgaat

SEQ ID NO: 22 - protein, 10 aa, synthetic construct
GYTFTGYFMN

SEQ ID NO: 23 - DNA, 51 bp, synthetic construct
  source 1..51: mol_type = other DNA
cgaatccacccatatgacggggacaccttttacaaccagaaattccagggg

SEQ ID NO: 24 - protein, 17 aa, synthetic construct
RIHPYDGDTFYNQKFQG

SEQ ID NO: 25 - DNA, 27 bp, synthetic construct
  source 1..27: mol_type = other DNA
tatgatggttcccgtgcaatggactac

SEQ ID NO: 26 - protein, 9 aa, synthetic construct
YDGSRAMDY

SEQ ID NO: 27 - DNA, 45 bp, synthetic construct
  source 1..45: mol_type = other DNA
aaggctagccagagcgtgagttttgccggcacttcacttatgcat

SEQ ID NO: 28 - protein, 15 aa, synthetic construct
KASQSVSFAGTSLMH

SEQ ID NO: 29 - DNA, 21 bp, synthetic construct
  source 1..21: mol_type = other DNA
cgggctagcaacctggaggcc

SEQ ID NO: 30 - protein, 7 aa, synthetic construct
RASNLEA

SEQ ID NO: 31 - DNA, 27 bp, synthetic construct
  source 1..27: mol_type = other DNA
cagcagtctcgcgagtatccttataca

SEQ ID NO: 32 - protein, 9 aa, synthetic construct
QQSREYPYT

SEQ ID NO: 33 - DNA, 135 bp, synthetic construct
  source 1..135: mol_type = other DNA
acgaccactcctgcaccccgccctccgactccggccccaaccattgccagccagcccctgtccctgcggccggaagcctgcagaccggctgccggcggagccgtccatacccggggactggatttcgcctgcgat

SEQ ID NO: 34 - protein, 45 aa, synthetic construct
TTTPAPRPPTPAPTIASQPLSLRPEACRPAAGGAVHTRGLDFACD

SEQ ID NO: 35 - DNA, 36 bp, synthetic construct
  source 1..36: mol_type = other DNA
gaatctaagtacggacctccctgcccgccctgtcct

SEQ ID NO: 36 - protein, 12 aa, synthetic construct
ESKYGPPCPPCP

SEQ ID NO: 37 - DNA, 72 bp, synthetic construct
  source 1..72: mol_type = other DNA
atctatatctgggcaccactcgccggaacctgtggagtgctgctgctgtcccttgtgatcaccctgtactgc

SEQ ID NO: 38 - protein, 24 aa, synthetic construct
IYIWAPLAGTCGVLLLSLVITLYC

SEQ ID NO: 39 - DNA, 126 bp, synthetic construct
  source 1..126: mol_type = other DNA
aagcgcggacggaagaaactcttgtacatcttcaagcagccgttcatgcgccctgtgcaaaccacccaagaagaggacgggtgctcctgccggttcccggaagaggaagagggcggctgcgaactg

SEQ ID NO: 40 - protein, 42 aa, synthetic construct
KRGRKKLLYIFKQPFMRPVQTTQEEDGCSCRFPEEEEGGCEL

SEQ ID NO: 41 - DNA, 336 bp, synthetic construct
  source 1..336: mol_type = other DNA
cgcgtgaagttttcccggtccgccgacgctccggcgtaccagcaggggcaaaaccagctgtacaacgaacttaacctcggtcgccgggaagaatatgacgtgctggacaagcggcggggaagagatcccgagatgggtggaaagccgcggcggaagaaccctcaggagggcttgtacaacgagctgcaaaaggacaaaatggccgaagcctactccgagattggcatgaagggagagcgcagacgcgggaagggacacgatggactgtaccagggactgtcaaccgcgactaaggacacttacgacgccctgcacatgcaggccctgcccccgcgc

SEQ ID NO: 42 - protein, 112 aa, synthetic construct
RVKFSRSADAPAYQQGQNQLYNELNLGRREEYDVLDKRRGRDPEMGGKPRRKNPQEGLYNELQKDKMAEAYSEIGMKGERRRGKGHDGLYQGLSTATKDTYDALHMQALPPR

SEQ ID NO: 43 - DNA, 45 bp, synthetic construct
  source 1..45: mol_type = other DNA
ggcggaggaggttccggtggagggggatcagggggtggaggatcg

SEQ ID NO: 44 - protein, 15 aa, synthetic construct
GGGGSGGGGSGGGGS

SEQ ID NO: 45 - DNA, 375 bp, synthetic construct
  source 1..375: mol_type = other DNA
atggaagtgcagctcgtggagtccggaggcggagtcgtgcagccgggcagatccctgcgcctttcctgctcggcatccgggtttaccttctctggctacggtctgtcgtgggtcagacaggctccagggaagggcctggaatgggtggccatgatctcctcggggggttcgtacacctactacgccgactcagtgaagggccggttcgccatctcccgcgacaacgccaagaacaccctgttcctgcaaatggactcgctccggcctgaggacactggggtgtacttctgcgcgagacacggagatgacccagcttggttcgcctactggggacaaggcacccctgtgaccgtgtcctccgcgagcaccaaggga

SEQ ID NO: 46 - protein, 125 aa, synthetic construct
MEVQLVESGGGVVQPGRSLRLSCSASGFTFSGYGLSWVRQAPGKGLEWVAMISSGGSYTYYADSVKGRFAISRDNAKNTLFLQMDSLRPEDTGVYFCARHGDDPAWFAYWGQGTPVTVSSASTKG

SEQ ID NO: 47 - DNA, 336 bp, synthetic construct
  source 1..336: mol_type = other DNA
gacattcagctgacccagagcccctcaagcctgtccgcgagcgttggggaccgcgtgaccatcacctgttcggtgtcctcctccatctcctccaacaatctccattggtaccagcagaaaccggggaaagcccccaagccgtggatctacggaacctccaacctggctagcggagtgccgtcgaggttctcgggctccggatcagggactgactacactttcactatttcctccctgcaaccggaggacattgccacctactactgtcagcagtggtcgtcctacccctacatgtataccttcggtcaaggaaccaaggtcgagatcaagaggaca

SEQ ID NO: 48 - protein, 112 aa, synthetic construct; identical to SEQ ID NO: 4

SEQ ID NO: 49 - DNA, 372 bp, synthetic construct
  source 1..372: mol_type = other DNA
atgcaagtgcagctcgtgcagtccggagccgaggtcgtgaagccgggcgcatccgtcaagatttcctgcaaggcatccgggtacaccttcaccggctacttcatgaactgggtcaagcagagcccagggcagtccctggaatggatcgggaggatccacccgtacgacggcgataccttctacaaccagaagttccagggcaaagccaccctgacggtcgacaagtcgagcaacaccgcgcacatggaactgctgtcgctcacttcggaggacttcgccgtgtactactgcactagatacgatggttcgcgcgctatggactactggggacaaggcaccaccgtgaccgtgtcctccgcgagcaccaaggga

SEQ ID NO: 50 - protein, 124 aa, synthetic construct
MQVQLVQSGAEVVKPGASVKISCKASGYTFTGYFMNWVKQSPGQSLEWIGRIHPYDGDTFYNQKFQGKATLTVDKSSNTAHMELLSLTSEDFAVYYCTRYDGSRAMDYWGQGTTVTVSSASTKG

SEQ ID NO: 51 - DNA, 339 bp, synthetic construct
  source 1..339: mol_type = other DNA
gacattgtgctgacccagagcccccttagcctggccgtgagcttggggcaacccgccatcatctcctgtaaagcctcccagtccgtgtcctttgccggaacttcgctcatgcattggtaccaccagaaaccggggcagcaacccagactgctcatctaccgcgcgtccaacctggaagccggagtgccggacaggttctcgggctccggatcaaagactgacttcactctgactatttccccggtggaggctgaggacgcagccacctactactgtcagcagtcacgggagtacccctataccttcggtggaggaaccaagcttgagatcaagaggaca

SEQ ID NO: 52 - protein, 113 aa, synthetic construct; identical to SEQ ID NO: 8

SEQ ID NO: 53 - DNA, 1500 bp, synthetic construct
  source 1..1500: mol_type = other DNA
atgttgctgctcgtgaccagcctccttctgtgcgaacttccccaccccgcattcctgctgattcctatggaagtgcagctcgtggagtccggaggcggagtcgtgcagccgggcagatccctgcgcctttcctgctcggcatccgggtttaccttctctggctacggtctgtcgtgggtcagacaggctccagggaagggcctggaatgggtggccatgatctcctcggggggttcgtacacctactacgccgactcagtgaagggccggttcgccatctcccgcgacaacgccaagaacaccctgttcctgcaaatggactcgctccggcctgaggacactggggtgtacttctgcgcgagacacggagatgacccagcttggttcgcctactggggacaaggcacccctgtgaccgtgtcctccgcgagcaccaagggaggcggaggaggttccggtggagggggatcagggggtggaggatcggacattcagctgacccagagcccctcaagcctgtccgcgagcgttggggaccgcgtgaccatcacctgttcggtgtcctcctccatctcctccaacaatctccattggtaccagcagaaaccggggaaagcccccaagccgtggatctacggaacctccaacctggctagcggagtgccgtcgaggttctcgggctccggatcagggactgactacactttcactatttcctccctgcaaccggaggacattgccacctactactgtcagcagtggtcgtcctacccctacatgtataccttcggtcaaggaaccaaggtcgagatcaagaggacagcggccgcaacgaccactcctgcaccccgccctccgactccggccccaaccattgccagccagcccctgtccctgcggccggaagcctgcagaccggctgccggcggagccgtccatacccggggactggatttcgcctgcgatatctatatctgggcaccactcgccggaacctgtggagtgctgctgctgtcccttgtgatcaccctgtactgcaagcgcggacggaagaaactcttgtacatcttcaagcagccgttcatgcgccctgtgcaaaccacccaagaagaggacgggtgctcctgccggttcccggaagaggaagagggcggctgcgaactgcgcgtgaagttttcccggtccgccgacgctccggcgtaccagcaggggcaaaaccagctgtacaacgaacttaacctcggtcgccgggaagaatatgacgtgctggacaagcggcggggaagagatcccgagatgggtggaaagccgcggcggaagaaccctcaggagggcttgtacaacgagctgcaaaaggacaaaatggccgaagcctactccgagattggcatgaagggagagcgcagacgcgggaagggacacgatggactgtaccagggactgtcaaccgcgactaaggacacttacgacgccctgcacatgcaggccctgcccccgcgc

SEQ ID NO: 54 - protein, 500 aa, synthetic construct
MLLLVTSLLLCELPHPAFLLIPMEVQLVESGGGVVQPGRSLRLSCSASGFTFSGYGLSWVRQAPGKGLEWVAMISSGGSYTYYADSVKGRFAISRDNAKNTLFLQMDSLRPEDTGVYFCARHGDDPAWFAYWGQGTPVTVSSASTKGGGGGSGGGGSGGGGSDIQLTQSPSSLSASVGDRVTITCSVSSSISSNNLHWYQQKPGKAPKPWIYGTSNLASGVPSRFSGSGSGTDYTFTISSLQPEDIATYYCQQWSSYPYMYTFGQGTKVEIKRTAAATTTPAPRPPTPAPTIASQPLSLRPEACRPAAGGAVHTRGLDFACDIYIWAPLAGTCGVLLLSLVITLYCKRGRKKLLYIFKQPFMRPVQTTQEEDGCSCRFPEEEEGGCELRVKFSRSADAPAYQQGQNQLYNELNLGRREEYDVLDKRRGRDPEMGGKPRRKNPQEGLYNELQKDKMAEAYSEIGMKGERRRGKGHDGLYQGLSTATKDTYDALHMQALPPR

SEQ ID NO: 55 - DNA, 1500 bp, synthetic construct
  source 1..1500: mol_type = other DNA
atgttgctgctcgtgaccagcctccttctgtgcgaacttccccaccccgcattcctgctgattcctgacattcagctgacccagagcccctcaagcctgtccgcgagcgttggggaccgcgtgaccatcacctgttcggtgtcctcctccatctcctccaacaatctccattggtaccagcagaaaccggggaaagcccccaagccgtggatctacggaacctccaacctggctagcggagtgccgtcgaggttctcgggctccggatcagggactgactacactttcactatttcctccctgcaaccggaggacattgccacctactactgtcagcagtggtcgtcctacccctacatgtataccttcggtcaaggaaccaaggtcgagatcaagaggacaggcggaggaggttccggtggagggggatcagggggtggaggatcgatggaagtgcagctcgtggagtccggaggcggagtcgtgcagccgggcagatccctgcgcctttcctgctcggcatccgggtttaccttctctggctacggtctgtcgtgggtcagacaggctccagggaagggcctggaatgggtggccatgatctcctcggggggttcgtacacctactacgccgactcagtgaagggccggttcgccatctcccgcgacaacgccaagaacaccctgttcctgcaaatggactcgctccggcctgaggacactggggtgtacttctgcgcgagacacggagatgacccagcttggttcgcctactggggacaaggcacccctgtgaccgtgtcctccgcgagcaccaagggagcggccgcaacgaccactcctgcaccccgccctccgactccggccccaaccattgccagccagcccctgtccctgcggccggaagcctgcagaccggctgccggcggagccgtccatacccggggactggatttcgcctgcgatatctatatctgggcaccactcgccggaacctgtggagtgctgctgctgtcccttgtgatcaccctgtactgcaagcgcggacggaagaaactcttgtacatcttcaagcagccgttcatgcgccctgtgcaaaccacccaagaagaggacgggtgctcctgccggttcccggaagaggaagagggcggctgcgaactgcgcgtgaagttttcccggtccgccgacgctccggcgtaccagcaggggcaaaaccagctgtacaacgaacttaacctcggtcgccgggaagaatatgacgtgctggacaagcggcggggaagagatcccgagatgggtggaaagccgcggcggaagaaccctcaggagggcttgtacaacgagctgcaaaaggacaaaatggccgaagcctactccgagattggcatgaagggagagcgcagacgcgggaagggacacgatggactgtaccagggactgtcaaccgcgactaaggacacttacgacgccctgcacatgcaggccctgcccccgcgc

SEQ ID NO: 56 - protein, 500 aa, synthetic construct
MLLLVTSLLLCELPHPAFLLIPDIQLTQSPSSLSASVGDRVTITCSVSSSISSNNLHWYQQKPGKAPKPWIYGTSNLASGVPSRFSGSGSGTDYTFTISSLQPEDIATYYCQQWSSYPYMYTFGQGTKVEIKRTGGGGSGGGGSGGGGSMEVQLVESGGGVVQPGRSLRLSCSASGFTFSGYGLSWVRQAPGKGLEWVAMISSGGSYTYYADSVKGRFAISRDNAKNTLFLQMDSLRPEDTGVYFCARHGDDPAWFAYWGQGTPVTVSSASTKGAAATTTPAPRPPTPAPTIASQPLSLRPEACRPAAGGAVHTRGLDFACDIYIWAPLAGTCGVLLLSLVITLYCKRGRKKLLYIFKQPFMRPVQTTQEEDGCSCRFPEEEEGGCELRVKFSRSADAPAYQQGQNQLYNELNLGRREEYDVLDKRRGRDPEMGGKPRRKNPQEGLYNELQKDKMAEAYSEIGMKGERRRGKGHDGLYQGLSTATKDTYDALHMQALPPR

SEQ ID NO: 57 - DNA, 1401 bp, synthetic construct
  source 1..1401: mol_type = other DNA
atgttgctgctcgtgaccagcctccttctgtgcgaacttccccaccccgcattcctgctgattcctatggaagtgcagctcgtggagtccggaggcggagtcgtgcagccgggcagatccctgcgcctttcctgctcggcatccgggtttaccttctctggctacggtctgtcgtgggtcagacaggctccagggaagggcctggaatgggtggccatgatctcctcggggggttcgtacacctactacgccgactcagtgaagggccggttcgccatctcccgcgacaacgccaagaacaccctgttcctgcaaatggactcgctccggcctgaggacactggggtgtacttctgcgcgagacacggagatgacccagcttggttcgcctactggggacaaggcacccctgtgaccgtgtcctccgcgagcaccaagggaggcggaggaggttccggtggagggggatcagggggtggaggatcggacattcagctgacccagagcccctcaagcctgtccgcgagcgttggggaccgcgtgaccatcacctgttcggtgtcctcctccatctcctccaacaatctccattggtaccagcagaaaccggggaaagcccccaagccgtggatctacggaacctccaacctggctagcggagtgccgtcgaggttctcgggctccggatcagggactgactacactttcactatttcctccctgcaaccggaggacattgccacctactactgtcagcagtggtcgtcctacccctacatgtataccttcggtcaaggaaccaaggtcgagatcaagaggacagcggccgcagaatctaagtacggacctccctgcccgccctgtcctatctatatctgggcaccactcgccggaacctgtggagtgctgctgctgtcccttgtgatcaccctgtactgcaagcgcggacggaagaaactcttgtacatcttcaagcagccgttcatgcgccctgtgcaaaccacccaagaagaggacgggtgctcctgccggttcccggaagaggaagagggcggctgcgaactgcgcgtgaagttttcccggtccgccgacgctccggcgtaccagcaggggcaaaaccagctgtacaacgaacttaacctcggtcgccgggaagaatatgacgtgctggacaagcggcggggaagagatcccgagatgggtggaaagccgcggcggaagaaccctcaggagggcttgtacaacgagctgcaaaaggacaaaatggccgaagcctactccgagattggcatgaagggagagcgcagacgcgggaagggacacgatggactgtaccagggactgtcaaccgcgactaaggacacttacgacgccctgcacatgcaggccctgcccccgcgc

SEQ ID NO: 58 - protein, 467 aa, synthetic construct
MLLLVTSLLLCELPHPAFLLIPMEVQLVESGGGVVQPGRSLRLSCSASGFTFSGYGLSWVRQAPGKGLEWVAMISSGGSYTYYADSVKGRFAISRDNAKNTLFLQMDSLRPEDTGVYFCARHGDDPAWFAYWGQGTPVTVSSASTKGGGGGSGGGGSGGGGSDIQLTQSPSSLSASVGDRVTITCSVSSSISSNNLHWYQQKPGKAPKPWIYGTSNLASGVPSRFSGSGSGTDYTFTISSLQPEDIATYYCQQWSSYPYMYTFGQGTKVEIKRTAAAESKYGPPCPPCPIYIWAPLAGTCGVLLLSLVITLYCKRGRKKLLYIFKQPFMRPVQTTQEEDGCSCRFPEEEEGGCELRVKFSRSADAPAYQQGQNQLYNELNLGRREEYDVLDKRRGRDPEMGGKPRRKNPQEGLYNELQKDKMAEAYSEIGMKGERRRGKGHDGLYQGLSTATKDTYDALHMQALPPR

SEQ ID NO: 59 - DNA, 1401 bp, synthetic construct
  source 1..1401: mol_type = other DNA
atgttgctgctcgtgaccagcctccttctgtgcgaacttccccaccccgcattcctgctgattcctgacattcagctgacccagagcccctcaagcctgtccgcgagcgttggggaccgcgtgaccatcacctgttcggtgtcctcctccatctcctccaacaatctccattggtaccagcagaaaccggggaaagcccccaagccgtggatctacggaacctccaacctggctagcggagtgccgtcgaggttctcgggctccggatcagggactgactacactttcactatttcctccctgcaaccggaggacattgccacctactactgtcagcagtggtcgtcctacccctacatgtataccttcggtcaaggaaccaaggtcgagatcaagaggacaggcggaggaggttccggtggagggggatcagggggtggaggatcgatggaagtgcagctcgtggagtccggaggcggagtcgtgcagccgggcagatccctgcgcctttcctgctcggcatccgggtttaccttctctggctacggtctgtcgtgggtcagacaggctccagggaagggcctggaatgggtggccatgatctcctcggggggttcgtacacctactacgccgactcagtgaagggccggttcgccatctcccgcgacaacgccaagaacaccctgttcctgcaaatggactcgctccggcctgaggacactggggtgtacttctgcgcgagacacggagatgacccagcttggttcgcctactggggacaaggcacccctgtgaccgtgtcctccgcgagcaccaagggagcggccgcagaatctaagtacggacctccctgcccgccctgtcctatctatatctgggcaccactcgccggaacctgtggagtgctgctgctgtcccttgtgatcaccctgtactgcaagcgcggacggaagaaactcttgtacatcttcaagcagccgttcatgcgccctgtgcaaaccacccaagaagaggacgggtgctcctgccggttcccggaagaggaagagggcggctgcgaactgcgcgtgaagttttcccggtccgccgacgctccggcgtaccagcaggggcaaaaccagctgtacaacgaacttaacctcggtcgccgggaagaatatgacgtgctggacaagcggcggggaagagatcccgagatgggtggaaagccgcggcggaagaaccctcaggagggcttgtacaacgagctgcaaaaggacaaaatggccgaagcctactccgagattggcatgaagggagagcgcagacgcgggaagggacacgatggactgtaccagggactgtcaaccgcgactaaggacacttacgacgccctgcacatgcaggccctgcccccgcgc

SEQ ID NO: 60 - protein, 467 aa, synthetic construct
MLLLVTSLLLCELPHPAFLLIPDIQLTQSPSSLSASVGDRVTITCSVSSSISSNNLHWYQQKPGKAPKPWIYGTSNLASGVPSRFSGSGSGTDYTFTISSLQPEDIATYYCQQWSSYPYMYTFGQGTKVEIKRTGGGGSGGGGSGGGGSMEVQLVESGGGVVQPGRSLRLSCSASGFTFSGYGLSWVRQAPGKGLEWVAMISSGGSYTYYADSVKGRFAISRDNAKNTLFLQMDSLRPEDTGVYFCARHGDDPAWFAYWGQGTPVTVSSASTKGAAAESKYGPPCPPCPIYIWAPLAGTCGVLLLSLVITLYCKRGRKKLLYIFKQPFMRPVQTTQEEDGCSCRFPEEEEGGCELRVKFSRSADAPAYQQGQNQLYNELNLGRREEYDVLDKRRGRDPEMGGKPRRKNPQEGLYNELQKDKMAEAYSEIGMKGERRRGKGHDGLYQGLSTATKDTYDALHMQALPPR

SEQ ID NO: 61 - DNA, 1500 bp, synthetic construct
  source 1..1500: mol_type = other DNA
atgttgctgctcgtgaccagcctccttctgtgcgaacttccccaccccgcattcctgctgattcctatgcaagtgcagctcgtgcagtccggagccgaggtcgtgaagccgggcgcatccgtcaagatttcctgcaaggcatccgggtacaccttcaccggctacttcatgaactgggtcaagcagagcccagggcagtccctggaatggatcgggaggatccacccgtacgacggcgataccttctacaaccagaagttccagggcaaagccaccctgacggtcgacaagtcgagcaacaccgcgcacatggaactgctgtcgctcacttcggaggacttcgccgtgtactactgcactagatacgatggttcgcgcgctatggactactggggacaaggcaccaccgtgaccgtgtcctccgcgagcaccaagggaggcggaggaggttccggtggagggggatcagggggtggaggatcggacattgtgctgacccagagcccccttagcctggccgtgagcttggggcaacccgccatcatctcctgtaaagcctcccagtccgtgtcctttgccggaacttcgctcatgcattggtaccaccagaaaccggggcagcaacccagactgctcatctaccgcgcgtccaacctggaagccggagtgccggacaggttctcgggctccggatcaaagactgacttcactctgactatttccccggtggaggctgaggacgcagccacctactactgtcagcagtcacgggagtacccctataccttcggtggaggaaccaagcttgagatcaagaggacagcggccgcaacgaccactcctgcaccccgccctccgactccggccccaaccattgccagccagcccctgtccctgcggccggaagcctgcagaccggctgccggcggagccgtccatacccggggactggatttcgcctgcgatatctatatctgggcaccactcgccggaacctgtggagtgctgctgctgtcccttgtgatcaccctgtactgcaagcgcggacggaagaaactcttgtacatcttcaagcagccgttcatgcgccctgtgcaaaccacccaagaagaggacgggtgctcctgccggttcccggaagaggaagagggcggctgcgaactgcgcgtgaagttttcccggtccgccgacgctccggcgtaccagcaggggcaaaaccagctgtacaacgaacttaacctcggtcgccgggaagaatatgacgtgctggacaagcggcggggaagagatcccgagatgggtggaaagccgcggcggaagaaccctcaggagggcttgtacaacgagctgcaaaaggacaaaatggccgaagcctactccgagattggcatgaagggagagcgcagacgcgggaagggacacgatggactgtaccagggactgtcaaccgcgactaaggacacttacgacgccctgcacatgcaggccctgcccccgcgc

SEQ ID NO: 62 - protein, 500 aa, synthetic construct
MLLLVTSLLLCELPHPAFLLIPMQVQLVQSGAEVVKPGASVKISCKASGYTFTGYFMNWVKQSPGQSLEWIGRIHPYDGDTFYNQKFQGKATLTVDKSSNTAHMELLSLTSEDFAVYYCTRYDGSRAMDYWGQGTTVTVSSASTKGGGGGSGGGGSGGGGSDIVLTQSPLSLAVSLGQPAIISCKASQSVSFAGTSLMHWYHQKPGQQPRLLIYRASNLEAGVPDRFSGSGSKTDFTLTISPVEAEDAATYYCQQSREYPYTFGGGTKLEIKRTAAATTTPAPRPPTPAPTIASQPLSLRPEACRPAAGGAVHTRGLDFACDIYIWAPLAGTCGVLLLSLVITLYCKRGRKKLLYIFKQPFMRPVQTTQEEDGCSCRFPEEEEGGCELRVKFSRSADAPAYQQGQNQLYNELNLGRREEYDVLDKRRGRDPEMGGKPRRKNPQEGLYNELQKDKMAEAYSEIGMKGERRRGKGHDGLYQGLSTATKDTYDALHMQALPPR

SEQ ID NO: 63 - DNA, 1500 bp, synthetic construct
  source 1..1500: mol_type = other DNA
atgttgctgctcgtgaccagcctccttctgtgcgaacttccccaccccgcattcctgctgattcctgacattgtgctgacccagagcccccttagcctggccgtgagcttggggcaacccgccatcatctcctgtaaagcctcccagtccgtgtcctttgccggaacttcgctcatgcattggtaccaccagaaaccggggcagcaacccagactgctcatctaccgcgcgtccaacctggaagccggagtgccggacaggttctcgggctccggatcaaagactgacttcactctgactatttccccggtggaggctgaggacgcagccacctactactgtcagcagtcacgggagtacccctataccttcggtggaggaaccaagcttgagatcaagaggacaggcggaggaggttccggtggagggggatcagggggtggaggatcgatgcaagtgcagctcgtgcagtccggagccgaggtcgtgaagccgggcgcatccgtcaagatttcctgcaaggcatccgggtacaccttcaccggctacttcatgaactgggtcaagcagagcccagggcagtccctggaatggatcgggaggatccacccgtacgacggcgataccttctacaaccagaagttccagggcaaagccaccctgacggtcgacaagtcgagcaacaccgcgcacatggaactgctgtcgctcacttcggaggacttcgccgtgtactactgcactagatacgatggttcgcgcgctatggactactggggacaaggcaccaccgtgaccgtgtcctccgcgagcaccaagggagcggccgcaacgaccactcctgcaccccgccctccgactccggccccaaccattgccagccagcccctgtccctgcggccggaagcctgcagaccggctgccggcggagccgtccatacccggggactggatttcgcctgcgatatctatatctgggcaccactcgccggaacctgtggagtgctgctgctgtcccttgtgatcaccctgtactgcaagcgcggacggaagaaactcttgtacatcttcaagcagccgttcatgcgccctgtgcaaaccacccaagaagaggacgggtgctcctgccggttcccggaagaggaagagggcggctgcgaactgcgcgtgaagttttcccggtccgccgacgctccggcgtaccagcaggggcaaaaccagctgtacaacgaacttaacctcggtcgccgggaagaatatgacgtgctggacaagcggcggggaagagatcccgagatgggtggaaagccgcggcggaagaaccctcaggagggcttgtacaacgagctgcaaaaggacaaaatggccgaagcctactccgagattggcatgaagggagagcgcagacgcgggaagggacacgatggactgtaccagggactgtcaaccgcgactaaggacacttacgacgccctgcacatgcaggccctgcccccgcgc

SEQ ID NO: 64 - protein, 500 aa, synthetic construct
MLLLVTSLLLCELPHPAFLLIPDIVLTQSPLSLAVSLGQPAIISCKASQSVSFAGTSLMHWYHQKPGQQPRLLIYRASNLEAGVPDRFSGSGSKTDFTLTISPVEAEDAATYYCQQSREYPYTFGGGTKLEIKRTGGGGSGGGGSGGGGSMQVQLVQSGAEVVKPGASVKISCKASGYTFTGYFMNWVKQSPGQSLEWIGRIHPYDGDTFYNQKFQGKATLTVDKSSNTAHMELLSLTSEDFAVYYCTRYDGSRAMDYWGQGTTVTVSSASTKGAAATTTPAPRPPTPAPTIASQPLSLRPEACRPAAGGAVHTRGLDFACDIYIWAPLAGTCGVLLLSLVITLYCKRGRKKLLYIFKQPFMRPVQTTQEEDGCSCRFPEEEEGGCELRVKFSRSADAPAYQQGQNQLYNELNLGRREEYDVLDKRRGRDPEMGGKPRRKNPQEGLYNELQKDKMAEAYSEIGMKGERRRGKGHDGLYQGLSTATKDTYDALHMQALPPR

SEQ ID NO: 65 - DNA, 1401 bp, synthetic construct
  source 1..1401: mol_type = other DNA
atgttgctgctcgtgaccagcctccttctgtgcgaacttccccaccccgcattcctgctgattcctatgcaagtgcagctcgtgcagtccggagccgaggtcgtgaagccgggcgcatccgtcaagatttcctgcaaggcatccgggtacaccttcaccggctacttcatgaactgggtcaagcagagcccagggcagtccctggaatggatcgggaggatccacccgtacgacggcgataccttctacaaccagaagttccagggcaaagccaccctgacggtcgacaagtcgagcaacaccgcgcacatggaactgctgtcgctcacttcggaggacttcgccgtgtactactgcactagatacgatggttcgcgcgctatggactactggggacaaggcaccaccgtgaccgtgtcctccgcgagcaccaagggaggcggaggaggttccggtggagggggatcagggggtggaggatcggacattgtgctgacccagagcccccttagcctggccgtgagcttggggcaacccgccatcatctcctgtaaagcctcccagtccgtgtcctttgccggaacttcgctcatgcattggtaccaccagaaaccggggcagcaacccagactgctcatctaccgcgcgtccaacctggaagccggagtgccggacaggttctcgggctccggatcaaagactgacttcactctgactatttccccggtggaggctgaggacgcagccacctactactgtcagcagtcacgggagtacccctataccttcggtggaggaaccaagcttgagatcaagaggacagcggccgcagaatctaagtacggacctccctgcccgccctgtcctatctatatctgggcaccactcgccggaacctgtggagtgctgctgctgtcccttgtgatcaccctgtactgcaagcgcggacggaagaaactcttgtacatcttcaagcagccgttcatgcgccctgtgcaaaccacccaagaagaggacgggtgctcctgccggttcccggaagaggaagagggcggctgcgaactgcgcgtgaagttttcccggtccgccgacgctccggcgtaccagcaggggcaaaaccagctgtacaacgaacttaacctcggtcgccgggaagaatatgacgtgctggacaagcggcggggaagagatcccgagatgggtggaaagccgcggcggaagaaccctcaggagggcttgtacaacgagctgcaaaaggacaaaatggccgaagcctactccgagattggcatgaagggagagcgcagacgcgggaagggacacgatggactgtaccagggactgtcaaccgcgactaaggacacttacgacgccctgcacatgcaggccctgcccccgcgc

SEQ ID NO: 66 - protein, 467 aa, synthetic construct
MLLLVTSLLLCELPHPAFLLIPMQVQLVQSGAEVVKPGASVKISCKASGYTFTGYFMNWVKQSPGQSLEWIGRIHPYDGDTFYNQKFQGKATLTVDKSSNTAHMELLSLTSEDFAVYYCTRYDGSRAMDYWGQGTTVTVSSASTKGGGGGSGGGGSGGGGSDIVLTQSPLSLAVSLGQPAIISCKASQSVSFAGTSLMHWYHQKPGQQPRLLIYRASNLEAGVPDRFSGSGSKTDFTLTISPVEAEDAATYYCQQSREYPYTFGGGTKLEIKRTAAAESKYGPPCPPCPIYIWAPLAGTCGVLLLSLVITLYCKRGRKKLLYIFKQPFMRPVQTTQEEDGCSCRFPEEEEGGCELRVKFSRSADAPAYQQGQNQLYNELNLGRREEYDVLDKRRGRDPEMGGKPRRKNPQEGLYNELQKDKMAEAYSEIGMKGERRRGKGHDGLYQGLSTATKDTYDALHMQALPPR

SEQ ID NO: 67 - DNA, 1401 bp, synthetic construct
  source 1..1401: mol_type = other DNA
atgttgctgctcgtgaccagcctccttctgtgcgaacttccccaccccgcattcctgctgattcctgacattgtgctgacccagagcccccttagcctggccgtgagcttggggcaacccgccatcatctcctgtaaagcctcccagtccgtgtcctttgccggaacttcgctcatgcattggtaccaccagaaaccggggcagcaacccagactgctcatctaccgcgcgtccaacctggaagccggagtgccggacaggttctcgggctccggatcaaagactgacttcactctgactatttccccggtggaggctgaggacgcagccacctactactgtcagcagtcacgggagtacccctataccttcggtggaggaaccaagcttgagatcaagaggacaggcggaggaggttccggtggagggggatcagggggtggaggatcgatgcaagtgcagctcgtgcagtccggagccgaggtcgtgaagccgggcgcatccgtcaagatttcctgcaaggcatccgggtacaccttcaccggctacttcatgaactgggtcaagcagagcccagggcagtccctggaatggatcgggaggatccacccgtacgacggcgataccttctacaaccagaagttccagggcaaagccaccctgacggtcgacaagtcgagcaacaccgcgcacatggaactgctgtcgctcacttcggaggacttcgccgtgtactactgcactagatacgatggttcgcgcgctatggactactggggacaaggcaccaccgtgaccgtgtcctccgcgagcaccaagggagcggccgcagaatctaagtacggacctccctgcccgccctgtcctatctatatctgggcaccactcgccggaacctgtggagtgctgctgctgtcccttgtgatcaccctgtactgcaagcgcggacggaagaaactcttgtacatcttcaagcagccgttcatgcgccctgtgcaaaccacccaagaagaggacgggtgctcctgccggttcccggaagaggaagagggcggctgcgaactgcgcgtgaagttttcccggtccgccgacgctccggcgtaccagcaggggcaaaaccagctgtacaacgaacttaacctcggtcgccgggaagaatatgacgtgctggacaagcggcggggaagagatcccgagatgggtggaaagccgcggcggaagaaccctcaggagggcttgtacaacgagctgcaaaaggacaaaatggccgaagcctactccgagattggcatgaagggagagcgcagacgcgggaagggacacgatggactgtaccagggactgtcaaccgcgactaaggacacttacgacgccctgcacatgcaggccctgcccccgcgc

SEQ ID NO: 68 - protein, 467 aa, synthetic construct
MLLLVTSLLLCELPHPAFLLIPDIVLTQSPLSLAVSLGQPAIISCKASQSVSFAGTSLMHWYHQKPGQQPRLLIYRASNLEAGVPDRFSGSGSKTDFTLTISPVEAEDAATYYCQQSREYPYTFGGGTKLEIKRTGGGGSGGGGSGGGGSMQVQLVQSGAEVVKPGASVKISCKASGYTFTGYFMNWVKQSPGQSLEWIGRIHPYDGDTFYNQKFQGKATLTVDKSSNTAHMELLSLTSEDFAVYYCTRYDGSRAMDYWGQGTTVTVSSASTKGAAAESKYGPPCPPCPIYIWAPLAGTCGVLLLSLVITLYCKRGRKKLLYIFKQPFMRPVQTTQEEDGCSCRFPEEEEGGCELRVKFSRSADAPAYQQGQNQLYNELNLGRREEYDVLDKRRGRDPEMGGKPRRKNPQEGLYNELQKDKMAEAYSEIGMKGERRRGKGHDGLYQGLSTATKDTYDALHMQALPPR

SEQ ID NO: 69 - protein, 210 aa, synthetic construct
RIAWARTELLNVCMNAKHHKEKPGPEDKLHEQCRPWRKNACCSTNTSQEAHKDVSYLYRFNWNHCGEMAPACKRHFIQDTCLYECSPNLGPWIQQVDQSWRKERVLNVPLCKEDCEQWWEDCRTSYTCKSNWHKGWNWTSGFNKCAVGAACQPFHFYFPTPTVLCNEIWTHSYKVSNYSRGSGRCIQMWFDPAQGNPNEEVARFYAAAMS

SEQ ID NO: 70 - protein, 214 aa, synthetic construct
TMCSAQDRTDLLNVCMDAKHHKTKPGPEDKLHDQCSPWKKNACCTASTSQELHKDTSRLYNFNWDHCGKMEPACKRHFIQDTCLYECSPNLGPWIQQVNQSWRKERFLDVPLCKEDCQRWWEDCHTSHTCKSNWHRGWDWTSGVNKCPAGALCRTFESYFPTPAALCEGLWSHSYKVSNYSRGSGRCIQMWFDSAQGNPNEEVARFYAAAMHVN

SEQ ID NO: 71 - protein, 223 aa, synthetic construct
QPRSARARTDLLNVCMNAKHHKTQPSPEDELYGQCSPWKKNACCTASTSQELHKDTSRLYNFNWDHCGKMEPTCKRHFIQDSCLYECSPNLGPWIRQVNQSWRKERILNVPLCKEDCERWWEDCRTSYTCKSNWHKGWNWTSGINECPAGALCSTFESYFPTPAALCEGLWSHSFKVSNYSRGSGRCIQMWFDSAQGNPNEEVAKFYAAAMNAGAPSRGIIDS

SEQ ID NO: 72 - protein, 150 aa, synthetic construct
QPRSARARTDLLNVCMNAKHHKTQPSPEDELYGQVGAPQGPSPGSVPLDDLPGAEEPEYGGDGCGGERLSPVSSPPSAVPGRRMPAARPAPARSCTRTPPACTTLTGITVVRWNPPASATLSRTAVSMSAHPTWGPGSGRSTRAGAKSAF

SEQ ID NO: 73 - protein, 209 aa, synthetic construct
GDELLNICMNAKHHKRVPSPEDKLYEECIPWKDNACCTLTTSWEAHLDVSPLYNFSLFHCGLLMPGCRKHFIQAICFYECSPNLGPWIQPVGSLGWEVAPSGQGERVVNVPLCQEDCEEWWEDCRMSYTCKSNWRGGWDWSQGKNRCPKGAQCLPFSHYFPTPADLCEKTWSNSFKASPERRNSGRCLQKWFEPAQGNPNVAVARLFAS

SEQ ID NO: 74 - protein, 224 aa, synthetic construct
GDELLNICMNAKHHKRVPSPEDKLYEECIPWKDNACCTLTTSWEAHLDVSPLYNFSLFHCGLLMPGCRKHFIQAICFYECSPNLGPWIQPVAPSGQGERVVNVPLCQEDCEEWWEDCRMSYTCKSNWRGGWDWSQGKNRCPKGAQCLPFSHYFPTPADLCEKTWSNSFKASPERRNSGRCLQKWFEPAQGNPNVAVARLFASSAPSWELSYTIMVCSLFLPFLS

SEQ ID NO: 75 - DNA, 855 bp, synthetic construct
  source 1..855: mol_type = other DNA
atggctcagcggatgacaacacagctgctgctccttctagtgtgggtggctgtagtaggggaggctcagacatacccgtacgacgtgcccgactatgcctacccctacgacgtcccggactacgcgtacccttacgatgtcccagattacgccaggattgcatgggccaggactgagcttctcaatgtctgcatgaacgccaagcaccacaaggaaaagccaggccccgaggacaagttgcatgagcagtgtcgtccctggaggaagaatgcctgctgttctaccaacaccagccaggaagcccataaggatgtttcctacctatatagattcaactggaaccactgtggagagatggcacctgcctgcaaacggcatttcatccaggacacctgcctctacgagtgctcccccaacttggggccctggatacagcaggtggatcagagctggcgcaaagagcgggtactgaacgtgcccctgtgcaaagaggactgtgagcaatggtgggaagattgtcgcacctcctacacctgcaagagcaactggcacaagggctggaactggacttcagggtttaacaagtgcgcagtgggagctgcctgccaacctttccatttctacttccccacacccactgttctgtgcaatgaaatctggactcactcctacaaggtcagcaactacagccgagggagtggccgctgcatccagatgtggttcgacccagcccagggcaaccccaatgaggaggtggcgaggttctatgctgcagccatgagtggggctgggccctgggcagcctggcctttcctgcttagcctggccctaatgctgctgtggctgctcagctga

SEQ ID NO: 76 - protein, 284 aa, synthetic construct
MAQRMTTQLLLLLVWVAVVGEAQTYPYDVPDYAYPYDVPDYAYPYDVPDYARIAWARTELLNVCMNAKHHKEKPGPEDKLHEQCRPWRKNACCSTNTSQEAHKDVSYLYRFNWNHCGEMAPACKRHFIQDTCLYECSPNLGPWIQQVDQSWRKERVLNVPLCKEDCEQWWEDCRTSYTCKSNWHKGWNWTSGFNKCAVGAACQPFHFYFPTPTVLCNEIWTHSYKVSNYSRGSGRCIQMWFDPAQGNPNEEVARFYAAAMSGAGPWAAWPFLLSLALMLLWLLS

SEQ ID NO: 77 - DNA, 849 bp, synthetic construct
  source 1..849: mol_type = other DNA
atggtctggaaatggatgccacttctgctgcttctggtctgtgtagcctacccgtacgacgtgcccgactatgcctacccctacgacgtcccggactacgcgtacccttacgatgtcccagattacgccaccatgtgcagtgcccaggacaggactgatctcctcaatgtctgtatggatgccaagcaccacaagacaaagccaggtcctgaggacaagctgcatgaccaatgcagtccctggaagaagaatgcctgctgcacagccagcaccagccaggagctgcacaaggacacctcccgcctgtacaactttaactgggaccactgcggcaagatggagcccgcctgcaagcgccacttcatccaggacacctgtctctatgagtgctcacccaacctggggccctggatacagcaggtgaatcagagctggcgcaaagaacgcttcctggatgtgcccttatgcaaagaggactgtcagcgctggtgggaggattgtcacacctcccacacgtgcaagagcaactggcacagaggatgggactggacctcaggagttaacaagtgcccagctggggctctctgccgcacctttgagtcctacttccccactccagctgccctttgtgaaggcctctggagtcactcatacaaggtcagcaactacagccgagggagcggccgctgcatccagatgtggtttgattcagcccagggcaaccccaacgaggaagtggcgaggttctatgctgcagccatgcatgtgaatgctggtgagatgcttcatgggactgggggtctcctgctcagtctggccctgatgctgcaactctggctccttggctga

SEQ ID NO: 78 - protein, 282 aa, synthetic construct
MVWKWMPLLLLLVCVAYPYDVPDYAYPYDVPDYAYPYDVPDYATMCSAQDRTDLLNVCMDAKHHKTKPGPEDKLHDQCSPWKKNACCTASTSQELHKDTSRLYNFNWDHCGKMEPACKRHFIQDTCLYECSPNLGPWIQQVNQSWRKERFLDVPLCKEDCQRWWEDCHTSHTCKSNWHRGWDWTSGVNKCPAGALCRTFESYFPTPAALCEGLWSHSYKVSNYSRGSGRCIQMWFDSAQGNPNEEVARFYAAAMHVNAGEMLHGTGGLLLSLALMLQLWLLG

SEQ ID NO: 79 - DNA, 855 bp, synthetic construct
  source 1..855: mol_type = other DNA
atggacatggcctggcagatgatgcagctgctgcttctggctttggtgactgctgcggggagtgcctacccgtacgacgtgcccgactatgcctacccctacgacgtcccggactacgcgtacccttacgatgtcccagattacgcccagcccaggagtgcgcgggccaggacggacctgctcaatgtctgcatgaacgccaagcaccacaagacacagcccagccccgaggacgagctgtatggccagtgcagtccctggaagaagaatgcctgctgcacggccagcaccagccaggagctgcacaaggacacctcccgcctgtacaactttaactgggatcactgtggtaagatggaacccacctgcaagcgccactttatccaggacagctgtctctatgagtgctcacccaacctggggccctggatacggcaggtcaaccagagctggcgcaaagagcgcattctgaacgtgcccctgtgcaaagaggactgtgagcgctggtgggaggactgtcgcacctcctacacctgcaaaagcaactggcacaaaggctggaattggacctcagggattaatgagtgtccggccggggccctctgcagcacctttgagtcctacttccccactccagccgccctttgtgaaggcctctggagccactccttcaaggtcagcaactatagtcgagggagcggccgctgcatccagatgtggtttgactcagcccagggcaaccccaatgaggaggtggccaagttctatgctgcggccatgagtggggctgggccctgggcagcctggcctttcctgcttagcctggccctaatgctgctgtggctgctcagctga

SEQ ID NO: 80 - protein, 284 aa, synthetic construct
MDMAWQMMQLLLLALVTAAGSAYPYDVPDYAYPYDVPDYAYPYDVPDYAQPRSARARTDLLNVCMNAKHHKTQPSPEDELYGQCSPWKKNACCTASTSQELHKDTSRLYNFNWDHCGKMEPTCKRHFIQDSCLYECSPNLGPWIRQVNQSWRKERILNVPLCKEDCERWWEDCRTSYTCKSNWHKGWNWTSGINECPAGALCSTFESYFPTPAALCEGLWSHSFKVSNYSRGSGRCIQMWFDSAQGNPNEEVAKFYAAAMSGAGPWAAWPFLLSLALMLLWLLS

SEQ ID NO: 81 - DNA, 834 bp, synthetic construct
  source 1..834: mol_type = other DNA
atggcatgctggtggccgctcctgctagagctgtggacagtcatgcccacctgggcttacccgtacgacgtgcccgactatgcctacccctacgacgtcccggactacgcgtacccttacgatgtcccagattacgccggggacgagctgctcaacatctgcatgaatgccaaacaccacaagagagtgcccagcccagaagacaagctctatgaggagtgcatcccctggaaggacaatgcctgctgcaccctcacgacaagctgggaagcccatctggatgtatccccactctacaacttcagcctgtttcactgtggactgctgatgcctggctgtcggaagcacttcatccaggctatctgcttctatgagtgctccccaaacctggggccctggatacagccagtgggaagcctggggtgggaggtggccccgagtgggcagggagagcgagttgtgaatgtgccgctgtgccaggaggactgtgaggagtggtgggaagactgtcgcatgtcttacacatgcaaatccaactggcgtggtggctgggactggagtcaggggaagaaccgctgccccaaaggggcccagtgcctccctttctcccattacttccccaccccagctgacctgtgtgagaagacttggagcaattccttcaaagccagccctgagcgacggaacagtgggcggtgtctccagaagtggtttgagcctgctcagggcaaccccaatgtggccgtggcccgcctcttcgccagctctgccccatcctgggaactgtcctacaccatcatggtctgctccctgttcctgccgttcctttcctga

SEQ ID NO: 82 - protein, 277 aa, synthetic construct
MACWWPLLLELWTVMPTWAYPYDVPDYAYPYDVPDYAYPYDVPDYAGDELLNICMNAKHHKRVPSPEDKLYEECIPWKDNACCTLTTSWEAHLDVSPLYNFSLFHCGLLMPGCRKHFIQAICFYECSPNLGPWIQPVGSLGWEVAPSGQGERVVNVPLCQEDCEEWWEDCRMSYTCKSNWRGGWDWSQGKNRCPKGAQCLPFSHYFPTPADLCEKTWSNSFKASPERRNSGRCLQKWFEPAQGNPNVAVARLFASSAPSWELSYTIMVCSLFLPFLS

SEQ ID NO: 83 - DNA, 849 bp, synthetic construct
  source 1..849: mol_type = other DNA
atggctcacctgatgactgtgcagttgttgctcctggtgatgtggatggccgaatgtgctcagtccagagcttacccgtacgacgtgcccgactatgcctacccctacgacgtcccggactacgcgtacccttacgatgtcccagattacgccactcgggccaggactgaacttctcaatgtctgcatggatgccaaacaccacaaagaaaaaccgggccctgaggacaatttacacgaccagtgcagcccctggaagacgaattcctgctgttccacgaacacaagccaggaagcacataaggacatttcctacctgtaccggttcaactggaaccactgcggaactatgacatcggaatgcaaacggcactttatccaagacacctgcctctatgagtgttccccgaacttgggaccctggatacagcaggtggaccagagctggcgcaaagagcggatacttgatgttcccctgtgcaaagaggactgtcagcagtggtgggaggactgccagagctcttttacctgcaagagcaattggcacaagggatggaactggtcctcggggcataacgagtgtcctgtgggagcctcctgccatcccttcaccttctacttccccacatctgctgctctgtgtgaggaaatctggagtcactcctacaagctcagcaactacagtcgagggagcggccgctgcattcagatgtggttcgacccagcccagggcaaccccaacgaggaagtggcgaggttctatgccgaggccatgagtggagctgggtttcatgggacctggccactcttgtgcagcctgtccttagtgctgctctgggtgatcagctga

SEQ ID NO: 84 - protein, 282 aa, synthetic construct
MAHLMTVQLLLLVMWMAECAQSRAYPYDVPDYAYPYDVPDYAYPYDVPDYATRARTELLNVCMDAKHHKEKPGPEDNLHDQCSPWKTNSCCSTNTSQEAHKDISYLYRFNWNHCGTMTSECKRHFIQDTCLYECSPNLGPWIQQVDQSWRKERILDVPLCKEDCQQWWEDCQSSFTCKSNWHKGWNWSSGHNECPVGASCHPFTFYFPTSAALCEEIWSHSYKLSNYSRGSGRCIQMWFDPAQGNPNEEVARFYAEAMSGAGFHGTWPLLCSLSLVLLWVIS

SEQ ID NO: 85 - DNA, 837 bp, synthetic construct
  source 1..837: mol_type = other DNA
atggcctggaaacagacaccactcttgcttttggtctacatggtcacaacaggcagtggctacccgtacgacgtgcccgactatgcctacccctacgacgtcccggactacgcgtacccttacgatgtcccagattacgcccgggacagaacagacctactcaacgtttgcatggatgccaaacaccataagacaaagccgggccccgaggacaagctgcatgaccagtgtagtccatggaagaaaaatgcctgttgctcagtcaacaccagccaggagctacacaaggctgactcccgtctgtacttcaactgggatcactgtggcaagatggagcctgcctgtaagagtcacttcatccaagactcctgcctgtatgagtgctcccccaaccttgggccttggatacagcaagtggaccagagttggcgtaaagagcgtttcctggatgtgcccttatgcaaagaggactgtcaccagtggtgggaagcctgtcgtacctcctttacctgcaagagagactggcataaaggctgggactggtcctcaggcattaacaagtgcccaaacacagcaccctgtcacacgtttgagtactacttcccgacaccagccagcctttgcgagggtctctggagtcactcctacaaggtcagcaactacagcagagggagtggccgctgcatccagatgtggtttgactcaacccagggcaatccgaatgaggacgtggtgaagttttatgcttcctttatgacatctgggactgtgccccatgcagcagtacttcttgtgcccagcctggccccagtgctgtcattatggctccctggctga

SEQ ID NO: 86 - protein, 278 aa, synthetic construct
MAWKQTPLLLLVYMVTTGSGYPYDVPDYAYPYDVPDYAYPYDVPDYARDRTDLLNVCMDAKHHKTKPGPEDKLHDQCSPWKKNACCSVNTSQELHKADSRLYFNWDHCGKMEPACKSHFIQDSCLYECSPNLGPWIQQVDQSWRKERFLDVPLCKEDCHQWWEACRTSFTCKRDWHKGWDWSSGINKCPNTAPCHTFEYYFPTPASLCEGLWSHSYKVSNYSRGSGRCIQMWFDSTQGNPNEDVVKFYASFMTSGTVPHAAVLLVPSLAPVLSLWLPG

SEQ ID NO: 87 - DNA, 816 bp, synthetic construct
  source 1..816: mol_type = other DNA
atggcacagtggtggcagatcctcttggggttgtgggcagtcctacccaccttggcatacccgtacgacgtgcccgactatgcctacccctacgacgtcccggactacgcgtacccttacgatgtcccagattacgccggggacaaactgctcagcgtctgcatgaattccaagcgccacaagcaagaacctggcccagaagacgaactctaccaggagtgcaggccttgggaggacaatgcctgctgcacacgttccacaagttgggaagcccaccttgaggagcccttgctctttaacttcagcatgatgcactgtggactgctgaccccggcctgtcgcaagcacttcatccaggccatctgcttccatgagtgttcccccaacctggggccttggatacagccggtggtcccaaacgggcaggaagagcagcgggtttggggcgtgccgctgtgccaggaggattgtgaggactggtggcgagcctgccactcatctttgacttgtaaatccaactggctccatggctgggactggagtgaggagaagaaacactgccccgcacatgagccctgcctccctttttcgtatcacttccccaccccggatgacctgtgtgagaagatctggaacaacacattcaaggccagtcccgagcgcaggaacagtgggcggtgtctgcagaagtggtttgagcccacccttagcaaccccaacgtggaagtggccctccactttgccggctctgccttagccccacagctctcttacaccctcccagccttctctctgtgcctgttgttccatccctga

SEQ ID NO: 88 - protein, 271 aa, synthetic construct
MAQWWQILLGLWAVLPTLAYPYDVPDYAYPYDVPDYAYPYDVPDYAGDKLLSVCMNSKRHKQEPGPEDELYQECRPWEDNACCTRSTSWEAHLEEPLLFNFSMMHCGLLTPACRKHFIQAICFHECSPNLGPWIQPVVPNGQEEQRVWGVPLCQEDCEDWWRACHSSLTCKSNWLHGWDWSEEKKHCPAHEPCLPFSYHFPTPDDLCEKIWNNTFKASPERRNSGRCLQKWFEPTLSNPNVEVALHFAGSALAPQLSYTLPAFSLCLLFHP

SEQ ID NO: 89 - DNA, 23 bp, synthetic construct
  source 1..23: mol_type = other DNA
cctacctatatagattcaactgg

SEQ ID NO: 90 - DNA, 20 bp, synthetic construct
  source 1..20: mol_type = other DNA
gggagacactgcatgtggaa

SEQ ID NO: 91 - DNA, 20 bp, synthetic construct
  source 1..20: mol_type = other DNA
ttcagtacccgctctttgcg

SEQ ID NO: 92 - DNA, 20 bp, synthetic construct
  source 1..20: mol_type = other DNA
gctcagcggatgacaacaca

SEQ ID NO: 93 - DNA, 19 bp, synthetic construct
  source 1..19: mol_type = other DNA
cctggcccatgcaatcctt

SEQ ID NO: 94 - DNA, 23 bp, synthetic construct
  source 1..23: mol_type = other DNA
cctctggagtcactcatacaagg

SEQ ID NO: 95 - DNA, 20 bp, synthetic construct
  source 1..20: mol_type = other DNA
cctgggctgaatcaaaccac

SEQ ID NO: 96 - DNA, 21 bp, synthetic construct
  source 1..21: mol_type = other DNA
cgcaaagagcgcattctgaac

SEQ ID NO: 97 - DNA, 20 bp, synthetic construct
  source 1..20: mol_type = other DNA
ctgggctgagtcaaaccaca

SEQ ID NO: 98 - DNA, 21 bp, synthetic construct
  source 1..21: mol_type = other DNA
cgcaaagagcgcattctgaac

SEQ ID NO: 99 - DNA, 20 bp, synthetic construct
  source 1..20: mol_type = other DNA
ctgggctgagtcaaaccaca

SEQ ID NO: 100 - DNA, 19 bp, synthetic construct
  source 1..19: mol_type = other DNA
ctggctgtcggaagcactt

SEQ ID NO: 101 - DNA, 20 bp, synthetic construct
  source 1..20: mol_type = other DNA
ggcacattcacaactcgctc

SEQ ID NO: 102 - DNA, 756 bp, synthetic construct
  source 1..756: mol_type = other DNA
atggaagtgcagctcgtggagtccggaggcggagtcgtgcagccgggcagatccctgcgcctttcctgctcggcatccgggtttaccttctctggctacggtctgtcgtgggtcagacaggctccagggaagggcctggaatgggtggccatgatctcctcggggggttcgtacacctactacgccgactcagtgaagggccggttcgccatctcccgcgacaacgccaagaacaccctgttcctgcaaatggactcgctccggcctgaggacactggggtgtacttctgcgcgagacacggagatgacccagcttggttcgcctactggggacaaggcacccctgtgaccgtgtcctccgcgagcaccaagggaggcggaggaggttccggtggagggggatcagggggtggaggatcggacattcagctgacccagagcccctcaagcctgtccgcgagcgttggggaccgcgtgaccatcacctgttcggtgtcctcctccatctcctccaacaatctccattggtaccagcagaaaccggggaaagcccccaagccgtggatctacggaacctccaacctggctagcggagtgccgtcgaggttctcgggctccggatcagggactgactacactttcactatttcctccctgcaaccggaggacattgccacctactactgtcagcagtggtcgtcctacccctacatgtataccttcggtcaaggaaccaaggtcgagatcaagaggaca

SEQ ID NO: 103 - protein, 252 aa, synthetic construct
MEVQLVESGGGVVQPGRSLRLSCSASGFTFSGYGLSWVRQAPGKGLEWVAMISSGGSYTYYADSVKGRFAISRDNAKNTLFLQMDSLRPEDTGVYFCARHGDDPAWFAYWGQGTPVTVSSASTKGGGGGSGGGGSGGGGSDIQLTQSPSSLSASVGDRVTITCSVSSSISSNNLHWYQQKPGKAPKPWIYGTSNLASGVPSRFSGSGSGTDYTFTISSLQPEDIATYYCQQWSSYPYMYTFGQGTKVEIKRT

SEQ ID NO: 104 - DNA, 1434 bp, synthetic construct
  source 1..1434: mol_type = other DNA
atggaagtgcagctcgtggagtccggaggcggagtcgtgcagccgggcagatccctgcgcctttcctgctcggcatccgggtttaccttctctggctacggtctgtcgtgggtcagacaggctccagggaagggcctggaatgggtggccatgatctcctcggggggttcgtacacctactacgccgactcagtgaagggccggttcgccatctcccgcgacaacgccaagaacaccctgttcctgcaaatggactcgctccggcctgaggacactggggtgtacttctgcgcgagacacggagatgacccagcttggttcgcctactggggacaaggcacccctgtgaccgtgtcctccgcgagcaccaagggaggcggaggaggttccggtggagggggatcagggggtggaggatcggacattcagctgacccagagcccctcaagcctgtccgcgagcgttggggaccgcgtgaccatcacctgttcggtgtcctcctccatctcctccaacaatctccattggtaccagcagaaaccggggaaagcccccaagccgtggatctacggaacctccaacctggctagcggagtgccgtcgaggttctcgggctccggatcagggactgactacactttcactatttcctccctgcaaccggaggacattgccacctactactgtcagcagtggtcgtcctacccctacatgtataccttcggtcaaggaaccaaggtcgagatcaagaggacagcggccgcaacgaccactcctgcaccccgccctccgactccggccccaaccattgccagccagcccctgtccctgcggccggaagcctgcagaccggctgccggcggagccgtccatacccggggactggatttcgcctgcgatatctatatctgggcaccactcgccggaacctgtggagtgctgctgctgtcccttgtgatcaccctgtactgcaagcgcggacggaagaaactcttgtacatcttcaagcagccgttcatgcgccctgtgcaaaccacccaagaagaggacgggtgctcctgccggttcccggaagaggaagagggcggctgcgaactgcgcgtgaagttttcccggtccgccgacgctccggcgtaccagcaggggcaaaaccagctgtacaacgaacttaacctcggtcgccgggaagaatatgacgtgctggacaagcggcggggaagagatcccgagatgggtggaaagccgcggcggaagaaccctcaggagggcttgtacaacgagctgcaaaaggacaaaatggccgaagcctactccgagattggcatgaagggagagcgcagacgcgggaagggacacgatggactgtaccagggactgtcaaccgcgactaaggacacttacgacgccctgcacatgcaggccctgcccccgcgc

SEQ ID NO: 105 - protein, 478 aa, synthetic construct
MEVQLVESGGGVVQPGRSLRLSCSASGFTFSGYGLSWVRQAPGKGLEWVAMISSGGSYTYYADSVKGRFAISRDNAKNTLFLQMDSLRPEDTGVYFCARHGDDPAWFAYWGQGTPVTVSSASTKGGGGGSGGGGSGGGGSDIQLTQSPSSLSASVGDRVTITCSVSSSISSNNLHWYQQKPGKAPKPWIYGTSNLASGVPSRFSGSGSGTDYTFTISSLQPEDIATYYCQQWSSYPYMYTFGQGTKVEIKRTAAATTTPAPRPPTPAPTIASQPLSLRPEACRPAAGGAVHTRGLDFACDIYIWAPLAGTCGVLLLSLVITLYCKRGRKKLLYIFKQPFMRPVQTTQEEDGCSCRFPEEEEGGCELRVKFSRSADAPAYQQGQNQLYNELNLGRREEYDVLDKRRGRDPEMGGKPRRKNPQEGLYNELQKDKMAEAYSEIGMKGERRRGKGHDGLYQGLSTATKDTYDALHMQALPPR

SEQ ID NO: 106 - DNA, 81 bp, synthetic construct
  source 1..81: mol_type = other DNA
ttttgggtgctggtggtggttggtggagtcctggcttgctatagcttgctagtaacagtggcctttattattttctgggtg

SEQ ID NO: 107 - protein, 27 aa, synthetic construct
FWVLVVVGGVLACYSLLVTVAFIIFWV

SEQ ID NO: 108 - DNA, 123 bp, synthetic construct
  source 1..123: mol_type = other DNA
cgcagcaaacgcagccgcctgctgcatagcgattatatgaacatgaccccgcgccgcccgggcccgacccgcaaacattatcagccgtatgcgccgccgcgcgattttgcggcgtatcgcagc

SEQ ID NO: 109 - protein, 41 aa, synthetic construct
RSKRSRLLHSDYMNMTPRRPGPTRKHYQPYAPPRDFAAYRS

SEQ ID NO: 110 - DNA, 196 bp, synthetic construct
  source 1..196: mol_type = other DNA
cgtgcggttgccgccatcctgggcctgggcctggtgctggggctgctgggccccctggccatcctgctggccctgtacctgctccggagggaccagaggctgccccccgatgcccacaagccccctgggggaggcagtttccggacccccatccaagaggagcaggccgacgcccactccaccctggccaagatct

SEQ ID NO: 111 - protein, 65 aa, synthetic construct
RAVAAILGLGLVLGLLGPLAILLALYLLRRDQRLPPDAHKPPGGGSFRTPIQEEQADAHSTLAKI

SEQ ID NO: 112 - DNA, 350 bp, synthetic construct
  source 1..350: mol_type = other DNA
ccatccagtgtcgaccctggaggaagaatgcctgctgttctaccaacaccagccaggaagcccataaggatgtttcctacctatatagattcaactggaaccactgtggagagatggcacctgcctgcaaacggcatttcatccaggacacctgcctctacgagtgctcccccaacttggggccctggatccagcaggtatgcatggcttcctgcaggtacaagacctagcggagcagctgagctttccaggcatctctgcaggctgcaaccccagctccagttctattcggggctgagttgctgggattcttgaacctgagcccttcttttgtatcaaaatcacccagg

SEQ ID NO: 113 - DNA, 302 bp, synthetic construct
  source 1..302: mol_type = other DNA
ccatccagtgtcgaccctggaggaagaatgcctgctgttctaccaactggaaccactgtggagagatggcacctgcctgcaaacggcatttcatccaggacacctgcctctacgagtgctcccccaacttggggccctggatccagcaggtatgcatggcttcctgcaggtacaagacctagcggagcagctgagctttccaggcatctctgcaggctgcaaccccagctccagttctattcggggctgagttgctgggattcttgaacctgagcccttcttttgtatcaaaatcacccagg